European Patent Specification EP 4 392 560 B1, published March 11, 2026. Title: CONSTRUCTS AND METHODS FOR PREPARING CIRCULAR RNA. Applicant: Peking University. Application Not Yet Assigned. The sequence listing filed with the application follows.

SEQUENCE LISTING (15 sequences)

SEQ ID NO: 1 - RNA, 741 nt, Coxsackievirus B3
uuaaaacagccuguggguugaucccacccacaggcccauugggcgcuagcacucugguaucacgguaccuuugugcgccuguuuuauacccccucccccaacuguaacuuagaaguaacacacaccgaucaacagucagcguggcacaccagccacguuuugaucaagcacuucuguuaccccggacugaguaucaauagacugcucacgcgguugaaggagaaagcguucguuauccggccaacuacuucgaaaaaccuaguaacaccguggaaguugcagaguguuucgcucagcacuaccccaguguagaucaggucgaugagucaccgcauuccccacgggcgaccguggcgguggcugcguuggcggccugcccauggggaaacccaugggacgcucuaauacagacauggugcgaagagucuauugagcuaguugguaguccuccggccccugaaugcggcuaauccuaacugcggagcacacacccucaagccagagggcagugugucguaacgggcaacucugcagcggaaccgacuacuuuggguguccguguuucauuuuauuccuauacuggcugcuuauggugacaauugagagaucguuaccauauagcuauuggauuggccauccggugacuaauagagcuauuauauaucccuuuguuggguuuauaccacuuagcuugaaagagguuaaaacauuacaauucauuguuaaguugaauacagcaaa

SEQ ID NO: 2 - RNA, 385 nt, Artificial Sequence
  Synthetic Construct
uuaaaacagccuguggguugaucccacccacaggcccauugggcgcuagcacucugguaucacgguaccuuugugcgccuguuuuauacccccucccccaacuguaacuuagaaguaacacacaccgaucaacagucagcguggcacaccagccacguuuugaucaagcacuucuguuaccccggacugaguaucaauagacugcucacgcgguugaaggagaaagcguucguuauccggccaacuacuucgaaaaaccuaguaacaccguggaaguugcagaguguuucgcucagcacuaccccaguguagaucaggucgaugagucaccgcauuccccacgggcgaccguggcgguggcugcguuggcggccugcccauguuu

SEQ ID NO: 3 - RNA, 364 nt, Artificial Sequence
  Synthetic Construct
ggggaaacccaaacaugggacgcucuaauacagacauggugcgaagagucuauugagcuaguugguaguccuccggccccugaaugcggcuaauccuaacugcggagcacacacccucaagccagagggcagugugucguaacgggcaacucugcagcggaaccgacuacuuuggguguccguguuucauuuuauuccuauacuggcugcuuauggugacaauugagagaucguuaccauauagcuauuggauuggccauccggugacuaauagagcuauuauauaucccuuuguuggguuuauaccacuuagcuugaaagagguuaaaacauuacaauucauuguuaaguugaauacagcaaa

SEQ ID NO: 4 - RNA, 346 nt, Artificial Sequence
  Synthetic Construct
uuaaaacagccuguggguugaucccacccacaggcccauugggcgcuagcacucugguaucacgguaccuuugugcgccuguuuuauacccccucccccaacuguaacuuagaaguaacacacaccgaucaacagucagcguggcacaccagccacguuuugaucaagcacuucuguuaccccggacugaguaucaauagacugcucacgcgguugaaggagaaagcguucguuauccggccaacuacuucgaaaaaccuaguaacaccguggaaguugcagaguguuucgcucagcacuaccccaguguagaucaggucgaugagucaccgcauuccccacguuu

SEQ ID NO: 5 - RNA, 403 nt, Artificial Sequence
  Synthetic Construct
gggcgaccaaacguggcgguggcugcguuggcggccugcccauggggaaacccaugggacgcucuaauacagacauggugcgaagagucuauugagcuaguugguaguccuccggccccugaaugcggcuaauccuaacugcggagcacacacccucaagccagagggcagugugucguaacgggcaacucugcagcggaaccgacuacuuuggguguccguguuucauuuuauuccuauacuggcugcuuauggugacaauugagagaucguuaccauauagcuauuggauuggccauccggugacuaauagagcuauuauauaucccuuuguuggguuuauaccacuuagcuugaaagagguuaaaacauuacaauucauuguuaaguugaauacagcaaa

SEQ ID NO: 6 - DNA, 19 bp, Artificial Sequence
  Synthetic Construct
taatacgactcactatagg

SEQ ID NO: 7 - DNA, 717 bp, Artificial Sequence
  Synthetic Construct
atggtgagcaagggcgaggagctgttcaccggggtggtgcccatcctggtcgagctggacggcgacgtaaacggccacaagttcagcgtgtccggcgagggcgagggcgatgccacctacggcaagctgaccctgaagttcatctgcaccaccggcaagctgcccgtgccctggcccaccctcgtgaccaccctgacctacggcgtgcagtgcttcagccgctaccccgaccacatgaagcagcacgacttcttcaagtccgccatgcccgaaggctacgtccaggagcgcaccatcttcttcaaggacgacggcaactacaagacccgcgccgaggtgaagttcgagggcgacaccctggtgaaccgcatcgagctgaagggcatcgacttcaaggaggacggcaacatcctggggcacaagctggagtacaactacaacagccacaacgtctatatcatggccgacaagcagaagaacggcatcaaggtgaacttcaagatccgccacaacatcgaggacggcagcgtgcagctcgccgaccactaccagcagaacacccccatcggcgacggccccgtgctgctgcccgacaaccactacctgagcacccagtccgccctgagcaaagaccccaacgagaagcgcgatcacatggtcctgctggagttcgtgaccgccgccgggatcactctcggcatggacgagctgtacaag

SEQ ID NO: 8 - DNA, 24 bp, Artificial Sequence
  Synthetic Construct
gattacaaggatgacgacgataag

SEQ ID NO: 9 - DNA, 57 bp, Artificial Sequence
  Synthetic Construct
gctactaacttcagcctgctgaagcaggctggagacgtggaggagaaccctggacct

SEQ ID NO: 10 - DNA, 1582 bp, Artificial Sequence
  Synthetic Construct
taatacgactcactataggggaaacccaaacatgggacgctctaatacagacatggtgcgaagagtctattgagctagttggtagtcctccggcccctgaatgcggctaatcctaactgcggagcacacaccctcaagccagagggcagtgtgtcgtaacgggcaactctgcagcggaaccgactactttgggtgtccgtgtttcattttattcctatactggctgcttatggtgacaattgagagatcgttaccatatagctattggattggccatccggtgactaatagagctattatatatccctttgttgggtttataccacttagcttgaaagaggttaaaacattacaattcattgttaagttgaatacagcaaaactagtgccaccatggtgagcaagggcgaggagctgttcaccggggtggtgcccatcctggtcgagctggacggcgacgtaaacggccacaagttcagcgtgtccggcgagggcgagggcgatgccacctacggcaagctgaccctgaagttcatctgcaccaccggcaagctgcccgtgccctggcccaccctcgtgaccaccctgacctacggcgtgcagtgcttcagccgctaccccgaccacatgaagcagcacgacttcttcaagtccgccatgcccgaaggctacgtccaggagcgcaccatcttcttcaaggacgacggcaactacaagacccgcgccgaggtgaagttcgagggcgacaccctggtgaaccgcatcgagctgaagggcatcgacttcaaggaggacggcaacatcctggggcacaagctggagtacaactacaacagccacaacgtctatatcatggccgacaagcagaagaacggcatcaaggtgaacttcaagatccgccacaacatcgaggacggcagcgtgcagctcgccgaccactaccagcagaacacccccatcggcgacggccccgtgctgctgcccgacaaccactacctgagcacccagtccgccctgagcaaagaccccaacgagaagcgcgatcacatggtcctgctggagttcgtgaccgccgccgggatcactctcggcatggacgagctgtacaaggattacaaggatgacgacgataaggctactaacttcagcctgctgaagcaggctggagacgtggaggagaaccctggacctgggtttttaaaacagcctgtgggttgatcccacccacaggcccattgggcgctagcactctggtatcacggtacctttgtgcgcctgttttataccccctcccccaactgtaacttagaagtaacacacaccgatcaacagtcagcgtggcacaccagccacgttttgatcaagcacttctgttaccccggactgagtatcaatagactgctcacgcggttgaaggagaaagcgttcgttatccggccaactacttcgaaaaacctagtaacaccgtggaagttgcagagtgtttcgctcagcactaccccagtgtagatcaggtcgatgagtcaccgcattccccacgggcgaccgtggcggtggctgcgttggcggcctgcccatgttt

SEQ ID NO: 11 - DNA, 1582 bp, Artificial Sequence
  Synthetic Construct
taatacgactcactatagggcgaccaaacgtggcggtggctgcgttggcggcctgcccatggggaaacccatgggacgctctaatacagacatggtgcgaagagtctattgagctagttggtagtcctccggcccctgaatgcggctaatcctaactgcggagcacacaccctcaagccagagggcagtgtgtcgtaacgggcaactctgcagcggaaccgactactttgggtgtccgtgtttcattttattcctatactggctgcttatggtgacaattgagagatcgttaccatatagctattggattggccatccggtgactaatagagctattatatatccctttgttgggtttataccacttagcttgaaagaggttaaaacattacaattcattgttaagttgaatacagcaaaactagtgccaccatggtgagcaagggcgaggagctgttcaccggggtggtgcccatcctggtcgagctggacggcgacgtaaacggccacaagttcagcgtgtccggcgagggcgagggcgatgccacctacggcaagctgaccctgaagttcatctgcaccaccggcaagctgcccgtgccctggcccaccctcgtgaccaccctgacctacggcgtgcagtgcttcagccgctaccccgaccacatgaagcagcacgacttcttcaagtccgccatgcccgaaggctacgtccaggagcgcaccatcttcttcaaggacgacggcaactacaagacccgcgccgaggtgaagttcgagggcgacaccctggtgaaccgcatcgagctgaagggcatcgacttcaaggaggacggcaacatcctggggcacaagctggagtacaactacaacagccacaacgtctatatcatggccgacaagcagaagaacggcatcaaggtgaacttcaagatccgccacaacatcgaggacggcagcgtgcagctcgccgaccactaccagcagaacacccccatcggcgacggccccgtgctgctgcccgacaaccactacctgagcacccagtccgccctgagcaaagaccccaacgagaagcgcgatcacatggtcctgctggagttcgtgaccgccgccgggatcactctcggcatggacgagctgtacaaggattacaaggatgacgacgataaggctactaacttcagcctgctgaagcaggctggagacgtggaggagaaccctggacctgggtttttaaaacagcctgtgggttgatcccacccacaggcccattgggcgctagcactctggtatcacggtacctttgtgcgcctgttttataccccctcccccaactgtaacttagaagtaacacacaccgatcaacagtcagcgtggcacaccagccacgttttgatcaagcacttctgttaccccggactgagtatcaatagactgctcacgcggttgaaggagaaagcgttcgttatccggccaactacttcgaaaaacctagtaacaccgtggaagttgcagagtgtttcgctcagcactaccccagtgtagatcaggtcgatgagtcaccgcattccccacgttt

SEQ ID NO: 12 - RNA, 54 nt, Artificial Sequence
  Synthetic Construct
gagggcagaggaagucuucuaacaugcggugacguggaggagaaucccggcccu

SEQ ID NO: 13 - DNA, 67 bp, Artificial Sequence
  Synthetic Construct
caccgacgcaaccgccggacgggtacaaacccctttgggtttgtaccctgcgagattatgtctgtac

SEQ ID NO: 14 - DNA, 30 bp, Artificial Sequence
  Synthetic Construct
gtggctgcgttggcggcctgcccatgtttg

SEQ ID NO: 15 - DNA, 70 bp, Artificial Sequence
  Synthetic Construct
gtggctgcgttggcggcctgcccatgtttgggggggaaacccaaacatgggacgctctaatacagacatg